European Patent Application EP 4 365 195 A1, published May 8, 2024. Title: ANTIBODY AGAINST NUCLEOCAPSID PROTEIN OF SARS-CoV-2 AND USE OF SAME. Applicant: TAUNS Laboratories, Inc. The sequence listing filed with the application follows.

SEQUENCE LISTING (121 sequences)

SEQ ID NO: 1 - protein, 419 aa, SARS CORONAVIRUS 2
MSDNGPQNQRNAPRITFGGPSDSTGSNQNGERSGARSKQRRPQGLPNNTASWFTALTQHGKEDLKFPRGQGVPINTNSSPDDQIGYYRRATRRIRGGDGKMKDLSPRWYFYYLGTGPEAGLPYGANKDGIIWVATEGALNTPKDHIGTRNPANNAAIVLQLPQGTTLPKGFYAEGSRGGSQASSRSSSRSRNSSRNSTPGSSRGTSPARMAGNGGDAALALLLLDRLNQLESKMSGKGQQQQGQTVTKKSAAEASKKPRQKRTATKAYNVTQAFGRRGPEQTQGNFGDQELIRQGTDYKHWPQIAQFAPSASAFFGMSRIGMEVTPSGTWLTYTAAIKLDDKDPNFKDQVILLNKHIDAYKTFPPTEPKKDKKKKADETQALPQRQKKQQTVTLLPAADLDDFSKQLQQSMSSADSTQA

SEQ ID NO: 2 - protein, 8 aa, Mouse
GYIFTDFI

SEQ ID NO: 3 - protein, 8 aa, Mouse
ISTYYGDA

SEQ ID NO: 4 - protein, 14 aa, Mouse
ARGGDYDEFYAMDH

SEQ ID NO: 5 - protein, 11 aa, Mouse
QNLLDSDGKTY

SEQ ID NO: 6 - protein, 3 aa, Mouse
LVS

SEQ ID NO: 7 - protein, 9 aa, Mouse
CQGTHFPQT

SEQ ID NO: 8 - protein, 8 aa, Mouse
GYTFTDYS

SEQ ID NO: 9 - protein, 8 aa, Mouse
INTETNES

SEQ ID NO: 10 - protein, 16 aa, Mouse
GSPYYYGNSYDWYFDV

SEQ ID NO: 11 - protein, 6 aa, Mouse
ENIYST

SEQ ID NO: 12 - protein, 3 aa, Mouse
AAT

SEQ ID NO: 13 - protein, 9 aa, Mouse
QHFWGFPWT

SEQ ID NO: 14 - protein, 8 aa, Mouse
GYTLTDYS

SEQ ID NO: 15 - protein, 8 aa, Mouse
VNTETADP

SEQ ID NO: 16 - protein, 12 aa, Mouse
ARGYYYGNTHDY

SEQ ID NO: 17 - protein, 6 aa, Mouse
ENIYSN

SEQ ID NO: 18 - protein, 3 aa, Mouse
LAT

SEQ ID NO: 19 - protein, 9 aa, Mouse
QHFWGTPYT

SEQ ID NO: 20 - protein, 8 aa, Mouse
GYSFTDYT

SEQ ID NO: 21 - protein, 8 aa, Mouse
INPNHGGT

SEQ ID NO: 22 - protein, 16 aa, Mouse
ARSGNFITTVGGLLDY

SEQ ID NO: 23 - protein, 12 aa, Mouse
QSLLYSSTQKNY

SEQ ID NO: 24 - protein, 3 aa, Mouse
WAS

SEQ ID NO: 25 - protein, 9 aa, Mouse
QQYYSYPYT

SEQ ID NO: 26 - protein, 8 aa, Mouse
GYTFTNYG

SEQ ID NO: 27 - protein, 8 aa, Mouse
INTYTGEP

SEQ ID NO: 28 - protein, 12 aa, Mouse
ARNYANYNYFDY

SEQ ID NO: 29 - protein, 6 aa, Mouse
ENIYSS

SEQ ID NO: 30 - protein, 3 aa, Mouse
TAT

SEQ ID NO: 31 - protein, 9 aa, Mouse
QHFWGTPWT

SEQ ID NO: 32 - protein, 8 aa, Mouse
GYTFTDYG

SEQ ID NO: 33 - protein, 8 aa, Mouse
INTHTGEP

SEQ ID NO: 34 - protein, 16 aa, Mouse
ARRGLYYDYDGRGFVY

SEQ ID NO: 35 - protein, 6 aa, Mouse
ENIYGN

SEQ ID NO: 36 - protein, 3 aa, Mouse
TAT

SEQ ID NO: 37 - protein, 9 aa, Mouse
QHFWGTPWT

SEQ ID NO: 38 - protein, 8 aa, Mouse
GYPFTNYG

SEQ ID NO: 39 - protein, 8 aa, Mouse
INTNTGEP

SEQ ID NO: 40 - protein, 10 aa, Mouse
ARDDNFWFAY

SEQ ID NO: 41 - protein, 10 aa, Mouse
QSVSTSTYTY

SEQ ID NO: 42 - protein, 3 aa, Mouse
YAS

SEQ ID NO: 43 - protein, 9 aa, Mouse
QHTWDIPYT

SEQ ID NO: 44 - protein, 8 aa, Mouse
GYTFTNYG

SEQ ID NO: 45 - protein, 8 aa, Mouse
INTDTGEP

SEQ ID NO: 46 - protein, 12 aa, Mouse
ASSAYYGNWFAY

SEQ ID NO: 47 - protein, 6 aa, Mouse
ENIYSN

SEQ ID NO: 48 - protein, 3 aa, Mouse
VAT

SEQ ID NO: 49 - protein, 9 aa, Mouse
QHFWGTPWT

SEQ ID NO: 50 - protein, 8 aa, Mouse
GYTFTDYG

SEQ ID NO: 51 - protein, 8 aa, Mouse
INTDTGEP

SEQ ID NO: 52 - protein, 12 aa, Mouse
ASSAYHGNWFLY

SEQ ID NO: 53 - protein, 6 aa, Mouse
ENVYGN

SEQ ID NO: 54 - protein, 3 aa, Mouse
VAT

SEQ ID NO: 55 - protein, 9 aa, Mouse
QHFWGTPWT

SEQ ID NO: 56 - protein, 8 aa, Mouse
GYTFTNYG

SEQ ID NO: 57 - protein, 8 aa, Mouse
INTNTGEP

SEQ ID NO: 58 - protein, 10 aa, Mouse
ARDGNFWFAY

SEQ ID NO: 59 - protein, 10 aa, Mouse
QSISTSDYIY

SEQ ID NO: 60 - protein, 3 aa, Mouse
YAS

SEQ ID NO: 61 - protein, 9 aa, Mouse
QHSWEIPYT

SEQ ID NO: 62 - protein, 9 aa, Rabbit
GFDFSSQNY

SEQ ID NO: 63 - protein, 8 aa, Rabbit
IYTVSGET

SEQ ID NO: 64 - protein, 17 aa, Rabbit
ARSPVKRIGVDMTRLDL

SEQ ID NO: 65 - protein, 8 aa, Rabbit
QSVFSDNY

SEQ ID NO: 66 - protein, 3 aa, Rabbit
YAS

SEQ ID NO: 67 - protein, 10 aa, Rabbit
QGYYSGYINV

SEQ ID NO: 68 - protein, 8 aa, Rabbit
GFDFSSDI

SEQ ID NO: 69 - protein, 8 aa, Rabbit
IVIDTTTT

SEQ ID NO: 70 - protein, 6 aa, Rabbit
ARAFSL

SEQ ID NO: 71 - protein, 7 aa, Rabbit
ESVVVNY

SEQ ID NO: 72 - protein, 3 aa, Rabbit
QAS

SEQ ID NO: 73 - protein, 10 aa, Rabbit
QGGYSGNIFP

SEQ ID NO: 74 - protein, 9 aa, Rabbit
GFDLNNYQY

SEQ ID NO: 75 - protein, 8 aa, Rabbit
IYTDSYIT

SEQ ID NO: 76 - protein, 17 aa, Rabbit
ARDVYVGYAGYAYALNL

SEQ ID NO: 77 - protein, 8 aa, Rabbit
QSVYNNNL

SEQ ID NO: 78 - protein, 3 aa, Rabbit
KAS

SEQ ID NO: 79 - protein, 12 aa, Rabbit
LGGVDDDADPNT

SEQ ID NO: 80 - protein, 8 aa, Rabbit
GIDFTNYD

SEQ ID NO: 81 - protein, 9 aa, Rabbit
ILAGSSGGP

SEQ ID NO: 82 - protein, 13 aa, Rabbit
AGSGYRNSFYFGL

SEQ ID NO: 83 - protein, 7 aa, Rabbit
SVYGNNY

SEQ ID NO: 84 - protein, 3 aa, Rabbit
QAS

SEQ ID NO: 85 - protein, 12 aa, Rabbit
QGTYWSDDWYNV

SEQ ID NO: 86 - protein, 8 aa, Rabbit
GFDFSTSA

SEQ ID NO: 87 - protein, 8 aa, Rabbit
IDTGSGNT

SEQ ID NO: 88 - protein, 6 aa, Rabbit
ARDFVL

SEQ ID NO: 89 - protein, 7 aa, Rabbit
SVYDSQV

SEQ ID NO: 90 - protein, 3 aa, Rabbit
KAS

SEQ ID NO: 91 - protein, 10 aa, Rabbit
AGAYSGNVVA

SEQ ID NO: 92 - protein, 9 aa, Rabbit
GFDFSGDIA

SEQ ID NO: 93 - protein, 8 aa, Rabbit
IVVDTTTT

SEQ ID NO: 94 - protein, 6 aa, Rabbit
ARAFSL

SEQ ID NO: 95 - protein, 7 aa, Rabbit
ESVAVNY

SEQ ID NO: 96 - protein, 3 aa, Rabbit
ETS

SEQ ID NO: 97 - protein, 10 aa, Rabbit
QGGYSGNDFP

SEQ ID NO: 98 - protein, 9 aa, Rabbit
GFDLSHFFY

SEQ ID NO: 99 - protein, 8 aa, Rabbit
IETAGGST

SEQ ID NO: 100 - protein, 18 aa, Rabbit
ARSIYTGTYAAYAYALNL

SEQ ID NO: 101 - protein, 8 aa, Rabbit
KSVYNNNY

SEQ ID NO: 102 - protein, 3 aa, Rabbit
GAS

SEQ ID NO: 103 - protein, 11 aa, Rabbit
AGGYSTSSDNG

SEQ ID NO: 104 - protein, 9 aa, Rabbit
GFSFNNKHY

SEQ ID NO: 105 - protein, 8 aa, Rabbit
IYAGDGTT

SEQ ID NO: 106 - protein, 14 aa, Rabbit
ARGDYYSYGYAYDI

SEQ ID NO: 107 - protein, 6 aa, Rabbit
EDIYSL

SEQ ID NO: 108 - protein, 3 aa, Rabbit
SAS

SEQ ID NO: 109 - protein, 10 aa, Rabbit
QCTYYSSSYA

SEQ ID NO: 110 - protein, 8 aa, Rabbit
GFDFSSDV

SEQ ID NO: 111 - protein, 8 aa, Rabbit
IVIDTTTT

SEQ ID NO: 112 - protein, 6 aa, Rabbit
ARTFSL

SEQ ID NO: 113 - protein, 7 aa, Rabbit
ESVVVKY

SEQ ID NO: 114 - protein, 3 aa, Rabbit
QAS

SEQ ID NO: 115 - protein, 10 aa, Rabbit
QGGYSGNIFP

SEQ ID NO: 116 - protein, 9 aa, Rabbit
GFSFSSSYY

SEQ ID NO: 117 - protein, 9 aa, Rabbit
IYAGSSGNT

SEQ ID NO: 118 - protein, 9 aa, Rabbit
AGDEDYWDL

SEQ ID NO: 119 - protein, 6 aa, Rabbit
QNIYSN

SEQ ID NO: 120 - protein, 3 aa, Rabbit
GTS

SEQ ID NO: 121 - protein, 12 aa, Rabbit
QSAYYSSTSSWT